European Patent Application EP 4 545 571 A1, published April 30, 2025. Title: FUSION PROTEIN HAVING TRIPLE ACTIVITY AND USE THEREOF. Applicant: Shanghai Minwei Biotechnology Co., LTD. The sequence listing filed with the application follows.

SEQUENCE LISTING (23 sequences)

SEQ ID NO: 1 - protein, 181 aa, synthetic construct
  source 1..181: note = Wild type FGF21
HPIPDSSPLLQFGGQVRQRYLYTDDAQQTEAHLEIREDGTVGGAADQSPESLLQLKALKPGVIQILGVKTSRFLCQRPDGALYGSLHFDPEACSFRELLLEDGYNVYQSEAHGLPLHLPGNKSPHRDPAPRGPARFLPLPGLPPALPEPPGILAPQPPDVGSSDPLSMVGPSQGRSPSYAS

SEQ ID NO: 2 - protein, 181 aa, synthetic construct
  source 1..181: note = FGF21 mutant
HPIPDSSPLLQFGGQVRQVYLYTDDAQQTEAHLEIREDGTVGGAADQSPESLLQLKALKPGVIQILGVKTSRFLCQRPDGALYGSLHFDPEACSFRERLLEDGYNVYQSEAHGLPLHLPGNKSPHRDPAPRGPARFLPLPGLPPALPEPPGILAPQPPDVGSSDPLSMVGNSTGRSPSYAS

SEQ ID NO: 3 - protein, 424 aa, synthetic construct
  source 1..424: note = Fc-FGF21 mutant fusion protein
ESKYGPPCPPCPAPEAAGGPSVFLFPPKPKDTLMISRTPEVTCVVVDVSQEDPEVQFNWYVDGVEVHNAKTKPREEQFNSTYRVVSVLTVLHQDWLNGKEYKCKVSNKGLPSSIEKTISKAKGQPREPQVYTLPPSQEEMTKNQVSLTCLVKGFYPSDIAVEWESNGQPENNYKTTPPVLDSDGSFFLYSRLTVDKSRWQEGNVFSCSVMHEALHNHYTQKSLSLSLGGGGGSGGGGSGGGGSHPIPDSSPLLQFGGQVRQVYLYTDDAQQTEAHLEIREDGTVGGAADQSPESLLQLKALKPGVIQILGVKTSRFLCQRPDGALYGSLHFDPEACSFRERLLEDGYNVYQSEAHGLPLHLPGNKSPHRDPAPRGPARFLPLPGLPPALPEPPGILAPQPPDVGSSDPLSMVGNSTGRSPSYAS

SEQ ID NO: 4 - protein, 479 aa, synthetic construct
  source 1..479: note = 12C1-F fusion protein
YGEGTFTSDYSILLDKIAQKAFIEWLIAGGPSSGAPPPSGGGGSGGGGSGGGGSAESKYGPPCPPCPAPEAAGGPSVFLFPPKPKDTLMISRTPEVTCVVVDVSQEDPEVQFNWYVDGVEVHNAKTKPREEQFNSTYRVVSVLTVLHQDWLNGKEYKCKVSNKGLPSSIEKTISKAKGQPREPQVYTLPPSQEEMTKNQVSLTCLVKGFYPSDIAVEWESNGQPENNYKTTPPVLDSDGSFFLYSRLTVDKSRWQEGNVFSCSVMHEALHNHYTQKSLSLSLGGGGGSGGGGSGGGGSHPIPDSSPLLQFGGQVRQVYLYTDDAQQTEAHLEIREDGTVGGAADQSPESLLQLKALKPGVIQILGVKTSRFLCQRPDGALYGSLHFDPEACSFRERLLEDGYNVYQSEAHGLPLHLPGNKSPHRDPAPRGPARFLPLPGLPPALPEPPGILAPQPPDVGSSDPLSMVGNSTGRSPSYAS

SEQ ID NO: 5 - protein, 479 aa, synthetic construct
  source 1..479: note = 12C3-F fusion protein
YGEGTFTSDYSIYLDKIAQKAFIEWLIAGGPSSGAPPPSGGGGSGGGGSGGGGSAESKYGPPCPPCPAPEAAGGPSVFLFPPKPKDTLMISRTPEVTCVVVDVSQEDPEVQFNWYVDGVEVHNAKTKPREEQFNSTYRVVSVLTVLHQDWLNGKEYKCKVSNKGLPSSIEKTISKAKGQPREPQVYTLPPSQEEMTKNQVSLTCLVKGFYPSDIAVEWESNGQPENNYKTTPPVLDSDGSFFLYSRLTVDKSRWQEGNVFSCSVMHEALHNHYTQKSLSLSLGGGGGSGGGGSGGGGSHPIPDSSPLLQFGGQVRQVYLYTDDAQQTEAHLEIREDGTVGGAADQSPESLLQLKALKPGVIQILGVKTSRFLCQRPDGALYGSLHFDPEACSFRERLLEDGYNVYQSEAHGLPLHLPGNKSPHRDPAPRGPARFLPLPGLPPALPEPPGILAPQPPDVGSSDPLSMVGNSTGRSPSYAS

SEQ ID NO: 6 - protein, 479 aa, synthetic construct
  source 1..479: note = 12C11-F fusion protein
HGEGTFTSDYSIYLDKIAAKDFIEWLIAGGPSSGAPPPSGGGGSGGGGSGGGGSAESKYGPPCPPCPAPEAAGGPSVFLFPPKPKDTLMISRTPEVTCVVVDVSQEDPEVQFNWYVDGVEVHNAKTKPREEQFNSTYRVVSVLTVLHQDWLNGKEYKCKVSNKGLPSSIEKTISKAKGQPREPQVYTLPPSQEEMTKNQVSLTCLVKGFYPSDIAVEWESNGQPENNYKTTPPVLDSDGSFFLYSRLTVDKSRWQEGNVFSCSVMHEALHNHYTQKSLSLSLGGGGGSGGGGSGGGGSHPIPDSSPLLQFGGQVRQVYLYTDDAQQTEAHLEIREDGTVGGAADQSPESLLQLKALKPGVIQILGVKTSRFLCQRPDGALYGSLHFDPEACSFRERLLEDGYNVYQSEAHGLPLHLPGNKSPHRDPAPRGPARFLPLPGLPPALPEPPGILAPQPPDVGSSDPLSMVGNSTGRSPSYAS

SEQ ID NO: 7 - protein, 479 aa, synthetic construct
  source 1..479: note = 12C12-F fusion protein
HSEGTFTSDYSILLDKIAQKAFIEWLIAGGPSSGAPPPSGGGGSGGGGSGGGGSAESKYGPPCPPCPAPEAAGGPSVFLFPPKPKDTLMISRTPEVTCVVVDVSQEDPEVQFNWYVDGVEVHNAKTKPREEQFNSTYRVVSVLTVLHQDWLNGKEYKCKVSNKGLPSSIEKTISKAKGQPREPQVYTLPPSQEEMTKNQVSLTCLVKGFYPSDIAVEWESNGQPENNYKTTPPVLDSDGSFFLYSRLTVDKSRWQEGNVFSCSVMHEALHNHYTQKSLSLSLGGGGGSGGGGSGGGGSHPIPDSSPLLQFGGQVRQVYLYTDDAQQTEAHLEIREDGTVGGAADQSPESLLQLKALKPGVIQILGVKTSRFLCQRPDGALYGSLHFDPEACSFRERLLEDGYNVYQSEAHGLPLHLPGNKSPHRDPAPRGPARFLPLPGLPPALPEPPGILAPQPPDVGSSDPLSMVGNSTGRSPSYAS

SEQ ID NO: 8 - protein, 39 aa, synthetic construct
  source 1..39: note = 12C1
YGEGTFTSDYSILLDKIAQKAFIEWLIAGGPSSGAPPPS

SEQ ID NO: 9 - protein, 39 aa, synthetic construct
  source 1..39: note = 12C2
HSEGTFTSDYSIYLDKIAQKAFIEWLIAGGPSSGAPPPS

SEQ ID NO: 10 - protein, 39 aa, synthetic construct
  source 1..39: note = 12C3
YGEGTFTSDYSIYLDKIAQKAFIEWLIAGGPSSGAPPPS

SEQ ID NO: 11 - protein, 39 aa, synthetic construct
  source 1..39: note = 12C4
HSEGTFTSDYSILLDKIAAKDFIEWLIAGGPSSGAPPPS

SEQ ID NO: 12 - protein, 39 aa, synthetic construct
  source 1..39: note = 12C5
YGEGTFTSDYSILLDKIAAKDFVQWLIAGGPSSGAPPPS

SEQ ID NO: 13 - protein, 39 aa, synthetic construct
  source 1..39: note = 12C6
HGEGTFTSDYSILLDKIAQKDFVQWLIAGGPSSGAPPPS

SEQ ID NO: 14 - protein, 39 aa, synthetic construct
  source 1..39: note = 12C7
HSEGTFTSDYSIYLDKIAAKDFIEWLIAGGPSSGAPPPS

SEQ ID NO: 15 - protein, 39 aa, synthetic construct
  source 1..39: note = 12C8
YGEGTFTSDYSIYLDKIAAKAFVQWLIAGGPSSGAPPPS

SEQ ID NO: 16 - protein, 39 aa, synthetic construct
  source 1..39: note = 12C9
HSEGTFTSDYSILLDKIAAKDFVQWLIAGGPSSGAPPPS

SEQ ID NO: 17 - protein, 39 aa, synthetic construct
  source 1..39: note = 12C10
YSEGTFTSDYSIYLDKIAAKAFVQWLIAGGPSSGAPPPS

SEQ ID NO: 18 - protein, 39 aa, synthetic construct
  source 1..39: note = 12C11
HGEGTFTSDYSIYLDKIAAKDFIEWLIAGGPSSGAPPPS

SEQ ID NO: 19 - protein, 39 aa, synthetic construct
  source 1..39: note = 12C12
HSEGTFTSDYSILLDKIAQKAFIEWLIAGGPSSGAPPPS

SEQ ID NO: 20 - protein, 39 aa, synthetic construct
  source 1..39: note = Polypeptide design template
  SITE 1: note = X =H or Y
  SITE 2: note = X =G or S
  SITE 13: note = X= Y or L
  SITE 19: note = X= A or Q
  SITE 21: note = X= A or D
  SITE 23: note = X= V or I
  SITE 24: note = X= A or Q or E
XXEGTFTSDYSIXLDKIAXKXFXXWLIAGGPSSGAPPPS

SEQ ID NO: 21 - protein, 228 aa, synthetic construct
  source 1..228: note = Fc
ESKYGPPCPPCPAPEAAGGPSVFLFPPKPKDTLMISRTPEVTCVVVDVSQEDPEVQFNWYVDGVEVHNAKTKPREEQFNSTYRVVSVLTVLHQDWLNGKEYKCKVSNKGLPSSIEKTISKAKGQPREPQVYTLPPSQEEMTKNQVSLTCLVKGFYPSDIAVEWESNGQPENNYKTTPPVLDSDGSFFLYSRLTVDKSRWQEGNVFSCSVMHEALHNHYTQKSLSLSLG

SEQ ID NO: 22 - protein, 16 aa, synthetic construct
  source 1..16: note = linker1
GGGGSGGGGSGGGGSA

SEQ ID NO: 23 - protein, 15 aa, synthetic construct
  source 1..15: note = linker2
GGGGSGGGGSGGGGS